European Patent Application EP 4 265 724 A1, published October 25, 2023. Title: RNA interference agent for inhibiting Hepatitis B virus expression and use thereof. Applicant: OliX Pharmaceuticals, Inc. The sequence listing filed with the application follows.

SEQUENCE LISTING (76 sequences)

SEQ ID NO: 1 - RNA, 16 nt, Artificial Sequence
  asiHBV-012 sense
gaugugucugcggcgu

SEQ ID NO: 2 - RNA, 19 nt, Artificial Sequence
  asiHBV-012 antisense
acgccgcagacacauccag

SEQ ID NO: 3 - RNA, 16 nt, Artificial Sequence
  asiHBV-014 sense
ugugucugcggcguuu

SEQ ID NO: 4 - RNA, 19 nt, Artificial Sequence
  asiHBV-014 antisense
aaacgccgcagacacaucc

SEQ ID NO: 5 - RNA, 16 nt, Artificial Sequence
  asiHBV-018 sense
gguauguugcccguuu

SEQ ID NO: 6 - RNA, 19 nt, Artificial Sequence
  asiHBV-018 antisense
aaacgggcaacauaccuug

SEQ ID NO: 7 - RNA, 16 nt, Artificial Sequence
  asiHBV-020 sense
gcccguuuguccucua

SEQ ID NO: 8 - RNA, 19 nt, Artificial Sequence
  asiHBV-020 antisense
uagaggacaaacgggcaac

SEQ ID NO: 9 - RNA, 16 nt, Artificial Sequence
  asiHBV-023 sense
aguuuacuagugccau

SEQ ID NO: 10 - RNA, 19 nt, Artificial Sequence
  asiHBV-023 antisense
auggcacuaguaaacugag

SEQ ID NO: 11 - RNA, 16 nt, Artificial Sequence
  asiHBV-027 sense
acuagugccauuuguu

SEQ ID NO: 12 - RNA, 19 nt, Artificial Sequence
  asiHBV-027 antisense
aacaaauggcacuaguaaa

SEQ ID NO: 13 - RNA, 16 nt, Artificial Sequence
  asiHBV-032 sense
uguucagugguucgua

SEQ ID NO: 14 - RNA, 19 nt, Artificial Sequence
  asiHBV-032 antisense
uacgaaccacugaacaaau

SEQ ID NO: 15 - RNA, 16 nt, Artificial Sequence
  asiHBV-033 sense
agugguucguagggcu

SEQ ID NO: 16 - RNA, 19 nt, Artificial Sequence
  asiHBV-033 antisense
agcccuacgaaccacugaa

SEQ ID NO: 17 - RNA, 16 nt, Artificial Sequence
  asiHBV-034 sense
gugguucguagggcuu

SEQ ID NO: 18 - RNA, 19 nt, Artificial Sequence
  asiHBV-034 antisense
aagcccuacgaaccacuga

SEQ ID NO: 19 - RNA, 16 nt, Artificial Sequence
  asiHBV-035 sense
ucaguuauauggauga

SEQ ID NO: 20 - RNA, 19 nt, Artificial Sequence
  asiHBV-035 antisense
ucauccauauaacugaaag

SEQ ID NO: 21 - RNA, 16 nt, Artificial Sequence
  asiHBV-039 sense
gcaccucucuuuacga

SEQ ID NO: 22 - RNA, 19 nt, Artificial Sequence
  asiHBV-039 antisense
ucguaaagagaggugcgcc

SEQ ID NO: 23 - RNA, 16 nt, Artificial Sequence
  asiHBV-040 sense
caccucucuuuacgca

SEQ ID NO: 24 - RNA, 19 nt, Artificial Sequence
  asiHBV-040 antisense
ugcguaaagagaggugcgc

SEQ ID NO: 25 - RNA, 16 nt, Artificial Sequence
  asiHBV-041 sense
accucucuuuacgcga

SEQ ID NO: 26 - RNA, 19 nt, Artificial Sequence
  asiHBV-041 antisense
ucgcguaaagagaggugcg

SEQ ID NO: 27 - RNA, 16 nt, Artificial Sequence
  asiHBV-043 sense
ccgucugugccuucua

SEQ ID NO: 28 - RNA, 19 nt, Artificial Sequence
  asiHBV-043 antisense
uagaaggcacagacgggga

SEQ ID NO: 29 - RNA, 16 nt, Artificial Sequence
  asiHBV-044 sense
cgucugugccuucuca

SEQ ID NO: 30 - RNA, 19 nt, Artificial Sequence
  asiHBV-044 antisense
ugagaaggcacagacgggg

SEQ ID NO: 31 - RNA, 16 nt, Artificial Sequence
  asiHBV-045 sense
gucugugccuucucau

SEQ ID NO: 32 - RNA, 19 nt, Artificial Sequence
  asiHBV-045 antisense
augagaaggcacagacggg

SEQ ID NO: 33 - RNA, 16 nt, Artificial Sequence
  asiHBV-046 sense
gugccuucucaucuga

SEQ ID NO: 34 - RNA, 19 nt, Artificial Sequence
  asiHBV-046 antisense
ucagaugagaaggcacaga

SEQ ID NO: 35 - RNA, 16 nt, Artificial Sequence
  asiHBV-049 sense
ccuucucaucugccga

SEQ ID NO: 36 - RNA, 19 nt, Artificial Sequence
  asiHBV-049 antisense
ucggcagaugagaaggcac

SEQ ID NO: 37 - RNA, 16 nt, Artificial Sequence
  asiHBV-056 sense
ugguggacuucucuca

SEQ ID NO: 38 - RNA, 19 nt, Artificial Sequence
  asiHBV-056 antisense
ugagagaaguccaccacga

SEQ ID NO: 39 - RNA, 16 nt, Artificial Sequence
  asiHBV-058 sense
gucugcggcguuuuau

SEQ ID NO: 40 - RNA, 19 nt, Artificial Sequence
  asiHBV-058 antisense
auaaaacgccgcagacaca

SEQ ID NO: 41 - RNA, 16 nt, Artificial Sequence
  asiHBV-059 sense
cugcggcguuuuauca

SEQ ID NO: 42 - RNA, 19 nt, Artificial Sequence
  asiHBV-059 antisense
ugauaaaacgccgcagaca

SEQ ID NO: 43 - RNA, 16 nt, Artificial Sequence
  asiHBV-060 sense
ugcggcguuuuaucau

SEQ ID NO: 44 - RNA, 19 nt, Artificial Sequence
  asiHBV-060 antisense
augauaaaacgccgcagac

SEQ ID NO: 45 - RNA, 16 nt, Artificial Sequence
  asiHBV-061 sense
cugcugcuaugccuca

SEQ ID NO: 46 - RNA, 19 nt, Artificial Sequence
  asiHBV-061 antisense
ugaggcauagcagcaggau

SEQ ID NO: 47 - RNA, 16 nt, Artificial Sequence
  asiHBV-062 sense
ugcugcuaugccucau

SEQ ID NO: 48 - RNA, 19 nt, Artificial Sequence
  asiHBV-062 antisense
augaggcauagcagcagga

SEQ ID NO: 49 - RNA, 16 nt, Artificial Sequence
  asiHBV-063 sense
cuaugccucaucuucu

SEQ ID NO: 50 - RNA, 19 nt, Artificial Sequence
  asiHBV-063 antisense
agaagaugaggcauagcag

SEQ ID NO: 51 - RNA, 16 nt, Artificial Sequence
  asiHBV-068 sense
uagugccauuuguuca

SEQ ID NO: 52 - RNA, 19 nt, Artificial Sequence
  asiHBV-068 antisense
ugaacaaauggcacuagua

SEQ ID NO: 53 - RNA, 16 nt, Artificial Sequence
  asiHBV-069 sense
ugguucguagggcuuu

SEQ ID NO: 54 - RNA, 19 nt, Artificial Sequence
  asiHBV-069 antisense
aaagcccuacgaaccacug

SEQ ID NO: 55 - RNA, 16 nt, Artificial Sequence
  asiHBV-072 sense
ccacggggcgcaccua

SEQ ID NO: 56 - RNA, 19 nt, Artificial Sequence
  asiHBV-072 antisense
uaggugcgccccguggucg

SEQ ID NO: 57 - RNA, 16 nt, Artificial Sequence
  asiHBV-073 sense
cacggggcgcaccucu

SEQ ID NO: 58 - RNA, 19 nt, Artificial Sequence
  asiHBV-073 antisense
agaggugcgccccgugguc

SEQ ID NO: 59 - RNA, 16 nt, Artificial Sequence
  asiHBV-074 sense
acggggcgcaccucua

SEQ ID NO: 60 - RNA, 19 nt, Artificial Sequence
  asiHBV-074 antisense
uagaggugcgccccguggu

SEQ ID NO: 61 - RNA, 16 nt, Artificial Sequence
  asiHBV-075 sense
cggggcgcaccucucu

SEQ ID NO: 62 - RNA, 19 nt, Artificial Sequence
  asiHBV-075 antisense
agagaggugcgccccgugg

SEQ ID NO: 63 - RNA, 16 nt, Artificial Sequence
  asiHBV-076 sense
ggggcgcaccucucuu

SEQ ID NO: 64 - RNA, 19 nt, Artificial Sequence
  asiHBV-076 antisense
aagagaggugcgccccgug

SEQ ID NO: 65 - RNA, 16 nt, Artificial Sequence
  asiHBV-080 sense
ucugugccuucucaua

SEQ ID NO: 66 - RNA, 19 nt, Artificial Sequence
  asiHBV-080 antisense
uaugagaaggcacagacgg

SEQ ID NO: 67 - RNA, 16 nt, Artificial Sequence
  asiHBV-082 sense
ugugccuucucaucua

SEQ ID NO: 68 - RNA, 19 nt, Artificial Sequence
  asiHBV-082 antisense
uagaugagaaggcacagac

SEQ ID NO: 69 - RNA, 16 nt, Artificial Sequence
  asiHBV-085 sense
ugccaacuggauccua

SEQ ID NO: 70 - RNA, 19 nt, Artificial Sequence
  asiHBV-085 antisense
uaggauccaguuggcagca

SEQ ID NO: 71 - RNA, 16 nt, Artificial Sequence
  asiHBV-086 sense
ugcugccaacuggaua

SEQ ID NO: 72 - RNA, 19 nt, Artificial Sequence
  asiHBV-086 antisense
uauccaguuggcagcacag

SEQ ID NO: 73 - RNA, 16 nt, Artificial Sequence
  asiHBV-103 sense
ugugccuucucaucua

SEQ ID NO: 74 - RNA, 21 nt, Artificial Sequence
  asiHBV-103 antisense
uagaugagaaggcacagacgg

SEQ ID NO: 75 - RNA, 17 nt, Artificial Sequence
  asiHBV-107 sense
cugugccuucucaucua

SEQ ID NO: 76 - RNA, 21 nt, Artificial Sequence
  asiHBV-107 antisense
uagaugagaaggcacagacgg